European Patent Application EP 4 112 648 A1, published January 4, 2023. Title: Anti- SARS-CoV-2-infection Protein and Vaccine. Applicant: WestVac Biopharma Co., Ltd. The sequence listing filed with the application follows.

SEQUENCE LISTING (20 sequences)

SEQ ID NO: 1 - protein, 223 aa, Artificial Sequence
RVQPTESIVRFPNITNLCPFGEVFNATRFASVYAWNRKRISNCVADYSVLYNSASFSTFKCYGVSPTKLNDLCFTNVYADSFVIRGDEVRQIAPGQTGKIADYNYKLPDDFTGCVIAWNSNNLDSKVGGNYNYLYRLFRKSNLKPFERDISTEIYQAGSTPCNGVEGFNCYFPLQSYGFQPTNGVGYQPYRVVVLSFELLHAPATVCGPKKSTNLVKNKCVNF

SEQ ID NO: 2 - protein, 222 aa, Artificial Sequence
VQPTESIVRFPNITNLCPFGEVFNATRFASVYAWNRKRISNCVADYSVLYNSASFSTFKCYGVSPTKLNDLCFTNVYADSFVIRGDEVRQIAPGQTGKIADYNYKLPDDFTGCVIAWNSNNLDSKVGGNYNYLYRLFRKSNLKPFERDISTEIYQAGSTPCNGVEGFNCYFPLQSYGFQPTNGVGYQPYRVVVLSFELLHAPATVCGPKKSTNLVKNKCVNF

SEQ ID NO: 3 - protein, 227 aa, Artificial Sequence
RVQPTESIVRFPNITNLCPFGEVFNATRFASVYAWNRKRISNCVADYSVLYNSASFSTFKCYGVSPTKLNDLCFTNVYADSFVIRGDEVRQIAPGQTGKIADYNYKLPDDFTGCVIAWNSNNLDSKVGGNYNYLYRLFRKSNLKPFERDISTEIYQAGSTPCNGVEGFNCYFPLQSYGFQPTNGVGYQPYRVVVLSFELLHAPATVCGPKKSTNLVKNKCVNFNFNG

SEQ ID NO: 4 - protein, 226 aa, Artificial Sequence
VQPTESIVRFPNITNLCPFGEVFNATRFASVYAWNRKRISNCVADYSVLYNSASFSTFKCYGVSPTKLNDLCFTNVYADSFVIRGDEVRQIAPGQTGKIADYNYKLPDDFTGCVIAWNSNNLDSKVGGNYNYLYRLFRKSNLKPFERDISTEIYQAGSTPCNGVEGFNCYFPLQSYGFQPTNGVGYQPYRVVVLSFELLHAPATVCGPKKSTNLVKNKCVNFNFNG

SEQ ID NO: 5 - protein, 274 aa, Artificial Sequence
MLLVNQSHQGFNKEHTSKMVSAIVLYVLLAAAAHSAFAADVQPTESIVRFPNITNLCPFGEVFNATRFASVYAWNRKRISNCVADYSVLYNSASFSTFKCYGVSPTKLNDLCFTNVYADSFVIRGDEVRQIAPGQTGKIADYNYKLPDDFTGCVIAWNSNNLDSKVGGNYNYLYRLFRKSNLKPFERDISTEIYQAGSTPCNGVEGFNCYFPLQSYGFQPTNGVGYQPYRVVVLSFELLHAPATVCGPKKSTNLVKNKCVNFNFNGHHHHHHHH

SEQ ID NO: 6 - protein, 395 aa, Artificial Sequence
MLLVNQSHQGFNKEHTSKMVSAIVLYVLLAAAAHSAFAADSDKIIHLTDDSFDTDVLKADGAILVDFWAEWCGPCKMIAPILDEIADEYQGKLTVAKLNIDQNPGTAPKYGIRGIPTLLLFKNGEVAATKVGALSKGQLKEFLDANLAGSGSGHMHHHHHHSSGDDDDKVQPTESIVRFPNITNLCPFGEVFNATRFASVYAWNRKRISNCVADYSVLYNSASFSTFKCYGVSPTKLNDLCFTNVYADSFVIRGDEVRQIAPGQTGKIADYNYKLPDDFTGCVIAWNSNNLDSKVGGNYNYLYRLFRKSNLKPFERDISTEIYQAGSTPCNGVEGFNCYFPLQSYGFQPTNGVGYQPYRVVVLSFELLHAPATVCGPKKSTNLVKNKCVNFNFNG

SEQ ID NO: 7 - protein, 394 aa, Artificial Sequence
MLLVNQSHQGFNKEHTSKMVSAIVLYVLLAAAAHSAFAADSIHIKDSDDLKNRLAEAGDKLVVIDFMATWCGPCKMIGPKLDEMANEMSDCIVVLKVDVDECEDIATEYNINSMPTFVFVKNSKKIEEFSGANVDKLRNTIIKLKLAGSGSGHMHHHHHHSSGDDDDKVQPTESIVRFPNITNLCPFGEVFNATRFASVYAWNRKRISNCVADYSVLYNSASFSTFKCYGVSPTKLNDLCFTNVYADSFVIRGDEVRQIAPGQTGKIADYNYKLPDDFTGCVIAWNSNNLDSKVGGNYNYLYRLFRKSNLKPFERDISTEIYQAGSTPCNGVEGFNCYFPLQSYGFQPTNGVGYQPYRVVVLSFELLHAPATVCGPKKSTNLVKNKCVNFNFNG

SEQ ID NO: 8 - DNA, 847 bp, Artificial Sequence
ggatccatgctgctggtcaaccaatctcatcagggcttcaacaaagaacatacttcaaaaatggtctccgctatcgtgctgtacgtgctcctcgctgctgctgctcactctgctttcgctgctgacgaattcagggtgcagccaaccgaatctatcgtcagattcccaaacatcactaacctgtgccctttcggagaggtgttcaacgctaccaggttcgccagcgtctacgcttggaaccgcaagcgtatcagcaactgcgtcgccgactactctgtgctgtacaactccgctagcttctctactttcaagtgctacggcgtgtcacctaccaagctgaacgacctgtgcttcactaacgtctacgccgactccttcgtgatccgcggagacgaagtccgtcagatcgctcctggacagaccggaaagatcgctgactacaactacaagctgccagacgacttcactggctgcgtgatcgcttggaactcaaacaacctggactccaaggtcggtggcaactacaactacctgtacaggctgttcagaaagtcaaacctgaagcctttcgagcgcgacatctcaaccgaaatctaccaggctggttccactccctgcaacggtgtggagggcttcaactgctacttccccctgcagtcctacggtttccagccaaccaacggagtcggttaccagccttaccgtgtggtcgtgctgagcttcgaactgctccacgctcctgctactgtgtgcggtcccaagaagtctactaacctggtcaaaaacaaatgtgtcaacttcaacttcaacggtcaccaccaccaccaccaccaccactgataagctt

SEQ ID NO: 9 - DNA, 1200 bp, Artificial Sequence
ggatccatgctgctggtcaaccagagccaccagggcttcaacaaggaacacacttccaagatggtgtccgccatcgtcctgtacgtgctgctggccgccgctgctcacagcgctttcgccgctgacagcgacaagatcatccacctgactgacgacagcttcgacactgacgtgctgaaggctgacggtgctatcctggtcgacttctgggccgagtggtgcggcccttgcaagatgatcgctcccatcctggacgagatcgccgacgagtaccagggtaaactgactgtggccaagctgaacatcgaccagaaccccggtactgctcctaagtacggcatccgtggtatccccactctgctgctgttcaagaacggtgaggtggccgctaccaaggtcggtgctctgagcaagggccagctgaaggagttcctggacgctaacctggctggttccggcagcggccacatgcaccaccaccaccatcacagcagcggcgacgacgacgacaaggtgcagccaaccgaatctatcgtcagattcccaaacatcactaacctgtgccctttcggagaggtgttcaacgctaccaggttcgccagcgtctacgcttggaaccgcaagcgtatcagcaactgcgtcgccgactactctgtgctgtacaactccgctagcttctctactttcaagtgctacggcgtgtcacctaccaagctgaacgacctgtgcttcactaacgtctacgccgactccttcgtgatccgcggagacgaagtccgtcagatcgctcctggacagaccggaaagatcgctgactacaactacaagctgccagacgacttcactggctgcgtgatcgcttggaactcaaacaacctggactccaaggtcggtggcaactacaactacctgtacaggctgttcagaaagtcaaacctgaagcctttcgagcgcgacatctcaaccgaaatctaccaggctggttccactccctgcaacggtgtggagggcttcaactgctacttccccctgcagtcctacggtttccagccaaccaacggagtcggttaccagccttaccgtgtggtcgtgctgagcttcgaactgctccacgctcctgctactgtgtgcggtcccaagaagtctactaacctggtcaaaaacaaatgtgtcaacttcaacttcaacggttaaaagctt

SEQ ID NO: 10 - DNA, 1197 bp, Artificial Sequence
ggatccatgctgctggtcaaccagagccaccagggtttcaacaaggaacacaccagcaagatggtgagcgctatcgtgctgtacgtcctgctggccgctgctgctcacagcgctttcgctgctgactccatccacatcaaggacagcgacgacctgaagaaccgtctggccgaggccggtgacaagctggtcgtcatcgacttcatggccacttggtgcggtccttgcaagatgatcggccctaagctggacgagatggctaacgagatgtccgactgcatcgtggtcctgaaggtggacgtcgacgagtgcgaggacatcgccaccgaatacaacatcaacagcatgcccaccttcgtgttcgtgaagaacagcaagaagatcgaggaattttccggcgctaacgtcgacaagctgcgtaacaccatcatcaagctgaagctggccggctccggctccggccacatgcatcaccaccaccaccattcctccggtgacgacgacgacaaggtgcagccaaccgaatctatcgtcagattcccaaacatcactaacctgtgccctttcggagaggtgttcaacgctaccaggttcgccagcgtctacgcttggaaccgcaagcgtatcagcaactgcgtcgccgactactctgtgctgtacaactccgctagcttctctactttcaagtgctacggcgtgtcacctaccaagctgaacgacctgtgcttcactaacgtctacgccgactccttcgtgatccgcggagacgaagtccgtcagatcgctcctggacagaccggaaagatcgctgactacaactacaagctgccagacgacttcactggctgcgtgatcgcttggaactcaaacaacctggactccaaggtcggtggcaactacaactacctgtacaggctgttcagaaagtcaaacctgaagcctttcgagcgcgacatctcaaccgaaatctaccaggctggttccactccctgcaacggtgtggagggcttcaactgctacttccccctgcagtcctacggtttccagccaaccaacggagtcggttaccagccttaccgtgtggtcgtgctgagcttcgaactgctccacgctcctgctactgtgtgcggtcccaagaagtctactaacctggtcaaaaacaaatgtgtcaacttcaacttcaacggttaaaagctt

SEQ ID NO: 11 - DNA, 711 bp, Artificial Sequence
aagcttgacgacgacgacaaggtgcagccgaccgaaagcattgtgcgctttccgaacattaccaacctttgtcctttcggtgaggtattcaatgcaacacgctttgcttcagtttatgcttggaaccgcaaacgcatttcaaactgtgttgctgattattcagttctttataactcagcttcattctccacctttaaatgttatggcgtttcacctacaaagctgaatgatctttgtttcaccaatgtttatgctgattcatttgttattcgcggcgatgaagttcgccagattgctcctggccagacaggcaagatagccgattataactataaacttcctgatgatttcacgggatgtgttattgcttggaactcaaacaaccttgattcaaaggtcggtggcaactataactatctttatcgcctgttccggaagtcaaaccttaaacctttcgagagagatatttcaacagaaatttatcaggctggctcaacaccttgtaacggcgttgaaggctttaactgttatttcccactgcaaagctatggctttcagcctacaaacggcgttggctatcagccttatcgcgttgttgttctttcatttgaacttcttcatgctcctgctacagtttgtggccctaagaaaagcactaatctggtgaaaaacaaatgtgtgaactttaactttaacggctgataactcgag

SEQ ID NO: 12 - DNA, 702 bp, Artificial Sequence
ctcgagaaaagagttcaacctacagaatcaatcgttagatttcctaacatcacaaacctttgtcctttcggcgaggtcttcaatgccacaagatttgcatcagtttatgcatggaacagaaagcgtatatcaaactgtgttgcagattattcagttctttataactcagcatcattctctacctttaaatgttatggagtttcacctacaaagctcaatgatctttgtttcactaatgtttatgcagattcatttgttatcagaggagatgaagttagacaaatcgcacctggacaaacaggaaagattgccgattataactataaacttcctgatgatttcaccggctgtgttatcgcatggaactcaaacaatctcgacagcaaagtaggtgggaattacaattacttgtaccggctatttaggaagtccaacctcaagccgttcgagcgcgatatctcaacagaaatctatcaagcaggatcaacaccttgtaacggagttgaaggatttaactgttatttcccgctacaatcatatggatttcaacctacaaacggagttggatatcaaccttatagagttgttgttctttcatttgaacttcttcatgcacctgcaacagtttgtggacctaagaagtctacgaaccttgttaagaataagtgtgttaactttaactttaacggatgataatctaga

SEQ ID NO: 13 - DNA, 807 bp, Artificial Sequence
atgaacagcttcagcaccagcgccttcggccccgtggccttcagcctgggcctgctgctggtgctgcccgccgccttccccgccccccaccaccaccaccaccaccaccacgacgacgacgacaaggtgcagcccaccgagagcatcgtgaggttccccaacatcaccaacctgtgccccttcggcgaggtgttcaacgccaccaggttcgccagcgtgtacgcctggaacaggaagaggatcagcaactgcgtggccgactacagcgtgctgtacaacagcgccagcttcagcaccttcaagtgctacggcgtgagccccaccaagctgaacgacctgtgcttcaccaacgtgtacgccgacagcttcgtgatcaggggcgacgaggtgaggcagatcgcccccggccagaccggcaagatcgccgactacaactacaagctgcccgacgacttcaccggctgcgtgatcgcctggaacagcaacaacctggacagcaaggtgggcggcaactacaactacctgtacaggctgttcaggaagagcaacctgaagcccttcgagagggacatcagcaccgagatctaccaggccggcagcaccccctgcaacggcgtggagggcttcaactgctacttccccctgcagagctacggcttccagcccaccaacggcgtgggctaccagccctacagggtggtggtgctgagcttcgagctgctgcacgcccccgccaccgtgtgcggccccaagaagagcaccaacctggtgaagaacaagtgcgtgaacttcaacttcaacggctga

SEQ ID NO: 14 - protein, 268 aa, Artificial Sequence
MNSFSTSAFGPVAFSLGLLLVLPAAFPAPHHHHHHHHDDDDKVQPTESIVRFPNITNLCPFGEVFNATRFASVYAWNRKRISNCVADYSVLYNSASFSTFKCYGVSPTKLNDLCFTNVYADSFVIRGDEVRQIAPGQTGKIADYNYKLPDDFTGCVIAWNSNNLDSKVGGNYNYLYRLFRKSNLKPFERDISTEIYQAGSTPCNGVEGFNCYFPLQSYGFQPTNGVGYQPYRVVVLSFELLHAPATVCGPKKSTNLVKNKCVNFNFNG

SEQ ID NO: 15 - DNA, 22 bp, Artificial Sequence
ggggaacttctcctgctagaat

SEQ ID NO: 16 - DNA, 22 bp, Artificial Sequence
cagacattttgctctcaagctg

SEQ ID NO: 17 - DNA, 20 bp, Artificial Sequence
ttgctgctgcttgacagatt

SEQ ID NO: 18 - DNA, 23 bp, Artificial Sequence
gctagagaacatctagacaagag

SEQ ID NO: 19 - DNA, 22 bp, Artificial Sequence
acacacgcatgacgacgttata

SEQ ID NO: 20 - DNA, 26 bp, Artificial Sequence
tgtgatcggtaggaatgacgcgaagc